European Patent Application EP 4 295 841 A2, published December 27, 2023. Title: SULFUR(VI) FLUORIDE COMPOUNDS AND METHODS FOR THE PREPARATION THEREOF. Applicant: THE SCRIPPS RESEARCH INSTITUTE. The sequence listing filed with the application follows.

SEQUENCE LISTING (12 sequences)

SEQ ID NO: 1 - protein, 6 aa, synthetic construct
  MOD_RES 6: note = AMIDATION
  MOD_RES 5: note = SULFATATION
DADEYL

SEQ ID NO: 2 - protein, 8 aa, synthetic construct
  MOD_RES 8: note = AMIDATION
  MOD_RES 3: note = SULFATATION
YEYLDYDF

SEQ ID NO: 3 - protein, 8 aa, synthetic construct
  MOD_RES 8: note = AMIDATION
  MOD_RES 1: note = SULFATATION
  MOD_RES 3: note = SULFATATION
  MOD_RES 6: note = SULFATATION
YEYLDYDF

SEQ ID NO: 4 - protein, 22 aa, synthetic construct
  MOD_RES 22: note = AMIDATION
  MOD_RES 5: note = SULFATATION
  MOD_RES 8: note = SULFATATION
TTPDYGHYDDKDTLDLNTPVDK

SEQ ID NO: 5 - protein, 20 aa, synthetic construct
  MOD_RES 20: note = AMIDATION
  MOD_RES 10..12: note = SULFATATION
  MOD_RES 14: note = SULFATATION
DADSENSSFYYYDYLDEVAF

SEQ ID NO: 6 - protein, 6 aa, synthetic construct
  MOD_RES 6: note = AMIDATION
  MOD_RES 5: note = Tyrosine-O-fluorosulfate
DADEYL

SEQ ID NO: 7 - protein, 12 aa, synthetic construct
  MOD_RES 12: note = AMIDATION
  MOD_RES 3: note = SULFATATION
GDYDSMKEPCFR

SEQ ID NO: 8 - protein, 12 aa, synthetic construct
  MOD_RES 12: note = AMIDATION
  MOD_RES 3: note = Tyrosine-O-fluorosulfate
GDYDSMKEPCFR

SEQ ID NO: 9 - protein, 8 aa, synthetic construct
  MOD_RES 7: note = Alpha-propargylglycine
  MOD_RES 5: note = Tyrosine-O-fluorosulfate
RKDVYGXG

SEQ ID NO: 10 - protein, 11 aa, synthetic construct
  REGION 1..6: note = Synthetically modified human hormone oxytocin, tyrosine-O-fluorosulfate, Xaa = alpha-propargylglycine
  MOD_RES 10: note = Alpha-propargylglycine
  MOD_RES 2: note = Tyrosine-O-fluorosulfate
  DISULFID 1..6: note = Disulfide bond
CYIQNCPLGXG

SEQ ID NO: 11 - protein, 11 aa, synthetic construct
  MOD_RES 10: note = Alpha-propargylglycine
  MOD_RES 2: note = Tyrosine-O-fluorosulfate
  DISULFID 1..6: note = Disulfide bond
CYFQNCPRGXG

SEQ ID NO: 12 - protein, 13 aa, synthetic construct
  MOD_RES 13: note = AMIDATION
  MOD_RES 2: note = Alpha-propargylglycine
  MOD_RES 8: note = Tyrosine-O-fluorosulfate
IXPWKWPYWPWRR